European Patent Application EP 4 656 658 A1, published December 3, 2025. Title: NEOADJUVANT IMMUNOTHERAPY WITH PD-L1 INHIBITOR IN TREATING CANCER. Applicant: ImmuneOncia Therapeutics, Inc. The sequence listing filed with the application follows.

SEQUENCE LISTING (10 sequences)

SEQ ID NO: 1 - protein, 121 aa, synthetic construct
  source 1..121: note = heavy chain (VH) variable domain of anti-PD-L1 antibody (IMC-001)
QMQLVQSGAEVKKPGSSVKVSCKASGGTFSSYAYSWVRQAPGQGLEWMGGIIPSFGTANYAQKFQGRVTITADESTSTAYMELSSLRSEDTAVYYCARGPIVATITPLDYWGQGTLVTVSS

SEQ ID NO: 2 - protein, 108 aa, synthetic construct
  source 1..108: note = light chain (VL) variable domain of anti-PD-L1 antibody (IMC-001)
SYVLTQPPSVSVAPGKTATIACGGENIGRKTVHWYQQKPGQAPVLVIYYDSDRPSGIPERFSGSNSGNTATLTISRVEAGDEADYYCLVWDSSSDHRIFGGGTKLTVL

SEQ ID NO: 3 - protein, 470 aa, synthetic construct
  source 1..470: note = heavy chain of anti-PD-L1 antibody (IMC-001)
MEWSWVFLFFLSVTTGVHSQMQLVQSGAEVKKPGSSVKVSCKASGGTFSSYAYSWVRQAPGQGLEWMGGIIPSFGTANYAQKFQGRVTITADESTSTAYMELSSLRSEDTAVYYCARGPIVATITPLDYWGQGTLVTVSSASTKGPSVFPLAPSSKSTSGGTAALGCLVKDYFPEPVTVSWNSGALTSGVHTFPAVLQSSGLYSLSSVVTVPSSSLGTQTYICNVNHKPSNTKVDKKVEPKSCDKTHTCPPCPAPELLGGPSVFLFPPKPKDTLMISRTPEVTCVVVDVSHEDPEVKFNWYVDGVEVHNAKTKPREEQYNSTYRVVSVLTVLHQDWLNGKEYKCKVSNKALPAPIEKTISKAKGQPREPQVYTLPPSRDELTKNQVSLTCLVKGFYPSDIAVEWESNGQPENNYKTTPPVLDSDGSFFLYSKLTVDKSRWQQGNVFSCSVMHEALHNHYTQKSLSLSPGK

SEQ ID NO: 4 - protein, 234 aa, synthetic construct
  source 1..234: note = light chain of anti-PD-L1 antibody (IMC-001)
MSVPTQVLGLLLLWLTDARCSYVLTQPPSVSVAPGKTATIACGGENIGRKTVHWYQQKPGQAPVLVIYYDSDRPSGIPERFSGSNSGNTATLTISRVEAGDEADYYCLVWDSSSDHRIFGGGTKLTVLGQPKAAPSVTLFPPSSEELQANKATLVCLISDFYPGAVTVAWKADSSPVKAGVETTTPSKQSNNKYAASSYLSLTPEQWKSHRSYSCQVTHEGSTVEKTVAPTECS

SEQ ID NO: 5 - protein, 5 aa, synthetic construct
  source 1..5: note = CDR1 (VH) of anti-PD-L1 antibody (IMC-001)
SYAYS

SEQ ID NO: 6 - protein, 17 aa, synthetic construct
  source 1..17: note = CDR2 (VH) of anti-PD-L1 antibody (IMC-001)
GIIPSFGTANYAQKFQG

SEQ ID NO: 7 - protein, 12 aa, synthetic construct
  source 1..12: note = CDR3 (VH) of anti-PD-L1 antibody (IMC-001)
GPIVATITPLDY

SEQ ID NO: 8 - protein, 11 aa, synthetic construct
  source 1..11: note = CDR1 (VL) of anti-PD-L1 antibody (IMC-001)
GGENIGRKTVH

SEQ ID NO: 9 - protein, 7 aa, synthetic construct
  source 1..7: note = CDR2 (VL) of anti-PD-L1 antibody (IMC-001)
YDSDRPS

SEQ ID NO: 10 - protein, 11 aa, synthetic construct
  source 1..11: note = CDR3 (VL) of anti-PD-L1 antibody (IMC-001)
LVWDSSSDHRI